European Patent Specification EP 3 653 728 B1, published February 1, 2023. Title: METHODS, SYSTEMS, COMPOSITIONS, KITS, APPARATUS AND COMPUTER-READABLE MEDIA FOR MOLECULAR TAGGING. Applicant: LIFE TECHNOLOGIES CORPORATION MONGAN, Ann CHIEN, Richard BRINZA, Dumitru BRAMLETT, Kelli. Application To Be Assigned. The sequence listing filed with the application follows.

SEQUENCE LISTING (2 sequences)

SEQ ID NO: 1 - DNA, 12 bp, Artificial Sequence
  Synthetic DNA
  misc_feature (1)..(9): where "N" represents any of A, T, C or G
nnnactnnntga

SEQ ID NO: 2 - DNA, 12 bp, Artificial Sequence
  Synthetic DNA
  misc_feature (1)..(9): where "N" represents any of A, T, C or G
nnnactnnntgc